European Patent Application EP 4 653 524 A1, published November 26, 2025. Title: FUNCTIONALITY-ENHANCED CELL THERAPY. Applicant: NANJING BIOHENG BIOTECH CO., LTD. Application EP. The sequence listing filed with the application follows.

SEQUENCE LISTING (82 sequences)

SEQ ID NO: 1 - protein, 7 aa, synthetic construct
  source 1..7: note = anti-Claudin18.2 CDR1-H
GSIFLIN

SEQ ID NO: 2 - protein, 5 aa, synthetic construct
  source 1..5: note = anti-Claudin18.2 CDR2-H
TRGGS

SEQ ID NO: 3 - protein, 14 aa, synthetic construct
  source 1..14: note = anti-Claudin18.2 CDR3-H
DLNLRSDPFKWYTF

SEQ ID NO: 4 - protein, 122 aa, synthetic construct
  source 1..122: note = anti-Claudin18.2 VHH
QVQLVESGGGLVQPGGSLRLSCAASGSIFLINAMGWYRQAPGKQRELVAVITRGGSANYTDSVKGRFTISRDNAKNTVYLQMNSLRAEDTAVYYCNADLNLRSDPFKWYTFWGQGTLVTVSS

SEQ ID NO: 5 - protein, 7 aa, synthetic construct
  source 1..7: note = anti-CD19 CDR1-H
GVSLPDY

SEQ ID NO: 6 - protein, 5 aa, synthetic construct
  source 1..5: note = anti-CD19 CDR2-H
WGSET

SEQ ID NO: 7 - protein, 12 aa, synthetic construct
  source 1..12: note = anti-CD19 CDR3-H
HYYYGGSYAMDY

SEQ ID NO: 8 - protein, 11 aa, synthetic construct
  source 1..11: note = anti-CD19 CDR1-L
RASQDISKYLN

SEQ ID NO: 9 - protein, 7 aa, synthetic construct
  source 1..7: note = anti-CD19 CDR2-L
HTSRLHS

SEQ ID NO: 10 - protein, 9 aa, synthetic construct
  source 1..9: note = anti-CD19 CDR3-L
QQGNTLPYT

SEQ ID NO: 11 - protein, 120 aa, synthetic construct
  source 1..120: note = anti-CD19 VH
QVTLKESGPVLVKPTETLTLTCTVSGVSLPDYGVSWIRQPPGKALEWLAVIWGSETTYYNSALKSRLTISKDTSKSQVVLTMTNMDPVDTATYYCARHYYYGGSYAMDYWGQGTMVTVSS

SEQ ID NO: 12 - protein, 106 aa, synthetic construct
  source 1..106: note = anti-CD19 VL
DIQMTQSPSSLSASVGDRVTITCRASQDISKYLNWYQQKPGKAPKLLLYHTSRLHSGVPSRFSGSGSGTDYTLTISSLQQEDFATYYCQQGNTLPYTFGQGTKVEI

SEQ ID NO: 13 - protein, 241 aa, synthetic construct
  source 1..241: note = anti-CD19 scFv
DIQMTQSPSSLSASVGDRVTITCRASQDISKYLNWYQQKPGKAPKLLLYHTSRLHSGVPSRFSGSGSGTDYTLTISSLQQEDFATYYCQQGNTLPYTFGQGTKVEIGGGGSGGGGSGGGGSQVTLKESGPVLVKPTETLTLTCTVSGVSLPDYGVSWIRQPPGKALEWLAVIWGSETTYYNSALKSRLTISKDTSKSQVVLTMTNMDPVDTATYYCARHYYYGGSYAMDYWGQGTMVTVSS

SEQ ID NO: 14 - protein, 27 aa, synthetic construct
  source 1..27: note = CD28 transmembrane domain
FWVLVVVGGVLACYSLLVTVAFIIFWV

SEQ ID NO: 15 - protein, 25 aa, synthetic construct
  source 1..25: note = CD8a transmembrane domain
IYIWAPLAGTCGVLLLSLVITLYCK

SEQ ID NO: 16 - protein, 21 aa, synthetic construct
  source 1..21: note = mCD8a transmembrane domain
IWAPLAGICVALLLSLIITLI

SEQ ID NO: 17 - protein, 41 aa, synthetic construct
  source 1..41: note = CD28 costimulatory domain
RSKRSRLLHSDYMNMTPRRPGPTRKHYQPYAPPRDFAAYRS

SEQ ID NO: 18 - protein, 40 aa, synthetic construct
  source 1..40: note = 4-1BB costimulatory domain
RGRKKLLYIFKQPFMRPVQTTQEEDGCSCRFPEEEEGGCE

SEQ ID NO: 19 - protein, 42 aa, synthetic construct
  source 1..42: note = m4-1BB costimulatory domain
RKKFPHIFKQPFKKTTGAAQEEDACSCRCPQEEEGGGGGYEL

SEQ ID NO: 20 - protein, 114 aa, synthetic construct
  source 1..114: note = CD3zm intracellular domain
LRVKFSRSADAPAYQQGQNQLFNELNLGRREEFDVLDKRRGRDPEMGGKPQRRKNPQEGLYNELQKDKMAEAYSEIGMKGERRRGKGHDGLFQGLSTATKDTFDALHMQALPPR

SEQ ID NO: 21 - protein, 113 aa, synthetic construct
  source 1..113: note = CD3z intracellular domain
LRVKFSRSADAPAYQQGQNQLYNELNLGRREEYDVLDKRRGRDPEMGGKPRRKNPQEGLYNELQKDKMAEAYSEIGMKGERRRGKGHDGLYQGLSTATKDTYDALHMQALPPR

SEQ ID NO: 22 - protein, 109 aa, synthetic construct
  source 1..109: note = mCD3z intracellular domain
SRSAETAANLQDPNQLYNELNLGRREEYDVLEKKRARDPEMGGKQQRRRNPQEGVYNALQKDKMAEAYSEIGTKGERRRGKGHDGLYQGLSTATKDTYDALHMQTLAPR

SEQ ID NO: 23 - protein, 20 aa, synthetic construct
  source 1..20: note = B2M signal peptide
MSRSVALAVLALLSLSGLEA

SEQ ID NO: 24 - protein, 21 aa, synthetic construct
  source 1..21: note = CD8a signal peptide
MALPVTALLLPLALLLHAARP

SEQ ID NO: 25 - protein, 24 aa, synthetic construct
  source 1..24: note = mCD8a signal peptide
MASPLTRFLSLNLLLLGESIILGS

SEQ ID NO: 26 - protein, 39 aa, synthetic construct
  source 1..39: note = CD28 hinge
IEVMYPPPYLDNEKSNGTIIHVKGKHLCPSPLFPGPSKP

SEQ ID NO: 27 - protein, 45 aa, synthetic construct
  source 1..45: note = CD8a hinge
TTTPAPRPPTPAPTIASQPLSLRPEACRPAAGGAVHTRGLDFACD

SEQ ID NO: 28 - protein, 45 aa, synthetic construct
  source 1..45: note = mCD8a hinge
TTTKPVLRTPSPVHPTGTSQPQRPEDCRPRGSVKGTGLDFACDIY

SEQ ID NO: 29 - protein, 12 aa, synthetic construct
  source 1..12: note = IgG4 hinge
ESKYGPPCPPCP

SEQ ID NO: 30 - protein, 18 aa, synthetic construct
  source 1..18: note = T2A
EGRGSLLTCGDVEENPGP

SEQ ID NO: 31 - protein, 15 aa, synthetic construct
  source 1..15: note = linker
GGGGSGGGGSGGGGS

SEQ ID NO: 32 - protein, 18 aa, synthetic construct
  source 1..18: note = linker
GSTSGSGKPGSGEGSTKG

SEQ ID NO: 33 - protein, 7 aa, synthetic construct
  source 1..7: note = anti-NKG2A CDR1-H
GFTFSSY

SEQ ID NO: 34 - protein, 6 aa, synthetic construct
  source 1..6: note = anti-NKG2A CDR2-H
SSGGSY

SEQ ID NO: 35 - protein, 10 aa, synthetic construct
  source 1..10: note = anti-NKG2A CDR3-H
HGDYPRFFDV

SEQ ID NO: 36 - protein, 11 aa, synthetic construct
  source 1..11: note = anti-NKG2A CDR1-L
SASSSVSSYIY

SEQ ID NO: 37 - protein, 7 aa, synthetic construct
  source 1..7: note = anti-NKG2A CDR2-L
LTSNLAS

SEQ ID NO: 38 - protein, 9 aa, synthetic construct
  source 1..9: note = anti-NKG2A CDR3-L
QQWSGNPYT

SEQ ID NO: 39 - protein, 119 aa, synthetic construct
  source 1..119: note = anti-NKG2A VH
EVQLVESGGGLVKPGGSLRLSCAASGFTFSSYAMSWVRQAPGKGLEWVAEISSGGSYTYYPDSVKGRFTISRDNAKNSLYLQMNSLRAEDTAVYYCTRHGDYPRFFDVWGQGTLVTVSS

SEQ ID NO: 40 - protein, 107 aa, synthetic construct
  source 1..107: note = anti-NKG2A VL
EIVLTQSPATLSLSPGERATMTCSASSSVSSYIYWYQQKPGQAPRLLIYLTSNLASGIPARFSGSGSGTDFTLTISSLEPEDFATYYCQQWSGNPYTFGQGTKVEIK

SEQ ID NO: 41 - protein, 244 aa, synthetic construct
  source 1..244: note = anti-NKG2A scFv
EIVLTQSPATLSLSPGERATMTCSASSSVSSYIYWYQQKPGQAPRLLIYLTSNLASGIPARFSGSGSGTDFTLTISSLEPEDFATYYCQQWSGNPYTFGQGTKVEIKGSTSGSGKPGSGEGSTKGEVQLVESGGGLVKPGGSLRLSCAASGFTFSSYAMSWVRQAPGKGLEWVAEISSGGSYTYYPDSVKGRFTISRDNAKNSLYLQMNSLRAEDTAVYYCTRHGDYPRFFDVWGQGTLVTVSS

SEQ ID NO: 42 - protein, 284 aa, synthetic construct
  source 1..284: note = HLA-E extracellular domain
GSHSLKYFHTSVSRPGRGEPRFISVGYVDDTQFVRFDNDAASPRMVPRAPWMEQEGSEYWDRETRSARDTAQIFRVNLRTLRGYYNQSEAGSHTLQWMHGCELGPDGRFLRGYEQFAYDGKDYLTLNEDLRSWTAVDTAAQISEQKSNDASEAEHQRAYLEDTCVEWLHKYLEKGKETLLHLEPPKTHVTHHPISDHEATLRCWALGFYPAEITLTWQQDGEGHTQDTELVETRPAGDGTFQKWAAVVVPSGEEQRYTCHVQHEGLPEPVTLRWKPASQPTIPI

SEQ ID NO: 43 - protein, 284 aa, synthetic construct
  source 1..284: note = HLA-E extracellular domain mutant
GSHSLKYFHTSVSRPGRGEPRFISVGYVDDTQFVRFDNDAASPRMVPRAPWMEQEGSEYWDRETRSARDTAQIFRVNLRTLRGCYNQSEAGSHTLQWMHGCELGPDGRFLRGYEQFAYDGKDYLTLNEDLRSWTAVDTAAQISEQKSNDASEAEHQRAYLEDTCVEWLHKYLEKGKETLLHLEPPKTHVTHHPISDHEATLRCWALGFYPAEITLTWQQDGEGHTQDTELVETRPAGDGTFQKWAAVVVPSGEEQRYTCHVQHEGLPEPVTLRWKPASQPTIPI

SEQ ID NO: 44 - protein, 7 aa, synthetic construct
  source 1..7: note = anti-PD1 CDR1-H
GYTFTNY

SEQ ID NO: 45 - protein, 6 aa, synthetic construct
  source 1..6: note = anti-PD1 CDR2-H
NPSNGG

SEQ ID NO: 46 - protein, 11 aa, synthetic construct
  source 1..11: note = anti-PD1 CDR3-H
RDYRFDMGFDY

SEQ ID NO: 47 - protein, 15 aa, synthetic construct
  source 1..15: note = anti-PD1 CDR1-L
RASKGVSTSGYSYLH

SEQ ID NO: 48 - protein, 7 aa, synthetic construct
  source 1..7: note = anti-PD1 CDR2-L
LASYLES

SEQ ID NO: 49 - protein, 9 aa, synthetic construct
  source 1..9: note = anti-PD1 CDR3-L
QHSRDLPLT

SEQ ID NO: 50 - protein, 120 aa, synthetic construct [sequence omitted]

SEQ ID NO: 51 - protein, 111 aa, synthetic construct [sequence omitted]

SEQ ID NO: 52 - protein, 246 aa, synthetic construct
  source 1..246: note = anti-PD1 scFv
QVQLVQSGVEVKKPGASVKVSCKASGYTFTNYYMYWVRQAPGQGLEWMGGINPSNGGTNFNEKFKNRVTLTTDSSTTTAYMELKSLQFDDTAVYYCARRDYRFDMGFDYWGQGTTVTVSSGGGGSGGGGSGGGGSEIVLTQSPATLSLSPGERATLSCRASKGVSTSGYSYLHWYQQKPGQAPRLLIYLASYLESGVPARFSGSGSGTDFTLTISSLEPEDFAVYYCQHSRDLPLTFGGGTKVEIK

SEQ ID NO: 53 - protein, 18 aa, synthetic construct
  source 1..18: note = PDL1 signal peptide
MRIFAVFIFMTYWHLLNA

SEQ ID NO: 54 - protein, 20 aa, synthetic construct
  source 1..20: note = PDL1 transmembrane domain
VILGAILLCLGVALTFIFRL

SEQ ID NO: 55 - protein, 223 aa, synthetic construct
  source 1..223: note = PDL1 extracellular domain
FTVTVPKDLYVVEYGSNMTIECKFPVEKQLDLAALIVYWEMEDKNIIQFVHGEEDLKVQHSSYRQRARLLKDQLSLGNAALQITDVKLQDAGVYRCMISYGGADYKRITVKVNAPYNKINQRILVVDPVTSEHELTCQAEGYPKAEVIWTSSDHQVLSGKTTTTNSKREEKLFNVTSTLRINTTTNEIFYCTFRRLDPEENHTAELVIPELPLAHPPNERTHL

SEQ ID NO: 56 - protein, 19 aa, synthetic construct
  source 1..19: note = PDL2 signal peptide
MIFLLLMLSLELQLHQIAA

SEQ ID NO: 57 - protein, 21 aa, synthetic construct
  source 1..21: note = PDL2 transmembrane domain
WLLHIFIPSCIIAFIFIATVI

SEQ ID NO: 58 - protein, 201 aa, synthetic construct
  source 1..201: note = PDL2 extracellular domain
LFTVTVPKELYIIEHGSNVTLECNFDTGSHVNLGAITASLQKVENDTSPHRERATLLEEQLPLGKASFHIPQVQVRDEGQYQCIIIYGVAWDYKYLTLKVKASYRKINTHILKVPETDEVELTCQATGYPLAEVSWPNVSVPANTSHSRTPEGLYQVTSVLRLKPPPGRNFSCVFWNTHVRELTLASIDLQSQMEPRTHPT

SEQ ID NO: 59 - protein, 7 aa, synthetic construct
  source 1..7: note = anti-FasL CDR1-H
GYIFISH

SEQ ID NO: 60 - protein, 6 aa, synthetic construct
  source 1..6: note = anti-FasL CDR2-H
NAYSGN

SEQ ID NO: 61 - protein, 11 aa, synthetic construct
  source 1..11: note = anti-FasL CDR3-H
ETMVRGVPCDY

SEQ ID NO: 62 - protein, 12 aa, synthetic construct
  source 1..12: note = anti-FasL CDR1-L
RASQSVSSSYLA

SEQ ID NO: 63 - protein, 7 aa, synthetic construct
  source 1..7: note = anti-FasL CDR2-L
GASSRAT

SEQ ID NO: 64 - protein, 9 aa, synthetic construct
  source 1..9: note = anti-FasL CDR3-L
QQYGSSPWT

SEQ ID NO: 65 - protein, 120 aa, synthetic construct
  source 1..120: note = anti-FasL VH
QVQLVQSGAEVKKPGASVKVSCKASGYIFISHGISWVRQAPGQGLEWMGWINAYSGNTNYAQKLQGRVTMTTDRSTSTAYMELRSLRSDDTAVYYCARETMVRGVPCDYWGQGTLVTVSS

SEQ ID NO: 66 - protein, 109 aa, synthetic construct
  source 1..109: note = anti-FasL VL
EIVLTQSPGTLSLSPGERATLSCRASQSVSSSYLAWYQQKPGQAPRLLIYGASSRATGIPDRFSGSGSGTDFTLTISRLEPEDFAVYYCQQYGSSPWTFGQGTKVEIKR

SEQ ID NO: 67 - protein, 244 aa, synthetic construct
  source 1..244: note = anti-FasL scFv
QVQLVQSGAEVKKPGASVKVSCKASGYIFISHGISWVRQAPGQGLEWMGWINAYSGNTNYAQKLQGRVTMTTDRSTSTAYMELRSLRSDDTAVYYCARETMVRGVPCDYWGQGTLVTVSSGGGGSGGGGSGGGGSEIVLTQSPGTLSLSPGERATLSCRASQSVSSSYLAWYQQKPGQAPRLLIYGASSRATGIPDRFSGSGSGTDFTLTISRLEPEDFAVYYCQQYGSSPWTFGQGTKVEIKR

SEQ ID NO: 68 - protein, 173 aa, synthetic construct
  source 1..173: note = Fas extracellular domain
MLGIWTLLPLVLTSVARLSSKSVNAQVTDINSKGLELRKTVTTVETQNLEGLHHDGQFCHKPCPPGERKARDCTVNGDEPDCVPCQEGKEYTDKAHFSSKCRRCRLCDEGHGLEVEINCTRTQNTKCRCKPNFFCNSTVCEHCDPCTKCEHGIIKECTLTSNTKCKEEGSRSN

SEQ ID NO: 69 - protein, 17 aa, synthetic construct
  source 1..17: note = Fas transmembrane domain
LGWLCLLLLPIPLIVWV

SEQ ID NO: 70 - protein, 7 aa, synthetic construct
  source 1..7: note = anti-CTLA4 CDR1-H
GFTFSSY

SEQ ID NO: 71 - protein, 6 aa, synthetic construct
  source 1..6: note = anti-CTLA4 CDR2-H
WYDGSN

SEQ ID NO: 72 - protein, 10 aa, synthetic construct
  source 1..10: note = anti-CTLA4 CDR3-H
APNYIGAFDV

SEQ ID NO: 73 - protein, 11 aa, synthetic construct
  source 1..11: note = anti-CTLA4 CDR1-L
RASQGISSWLA

SEQ ID NO: 74 - protein, 7 aa, synthetic construct
  source 1..7: note = anti-CTLA4 CDR2-L
AASSLQS

SEQ ID NO: 75 - protein, 9 aa, synthetic construct
  source 1..9: note = anti-CTLA4 CDR3-L
QQYNSYPPT

SEQ ID NO: 76 - protein, 119 aa, synthetic construct
  source 1..119: note = anti-CTLA4 VH
QVQLVESGGGVVQPGRSLRLSCAASGFTFSSYGMHWVRQAPGKGLEWVAVIWYDGSNKYYADSVKGRFTISRDNSKNTLYLQMNSLRAEDTAVFYCARAPNYIGAFDVWGQGTMVTVSS

SEQ ID NO: 77 - protein, 107 aa, synthetic construct
  source 1..107: note = anti-CTLA4 VL
DIQMTQSPSSLSASVGDRVTITCRASQGISSWLAWYQQKPEKAPKSLIYAASSLQSGVPSRFSGSGSGTDFTLTISSLQPEDFATYYCQQYNSYPPTFGQGTKVEIK

SEQ ID NO: 78 - protein, 241 aa, synthetic construct
  source 1..241: note = anti-CTLA4 scFv
QVQLVESGGGVVQPGRSLRLSCAASGFTFSSYGMHWVRQAPGKGLEWVAVIWYDGSNKYYADSVKGRFTISRDNSKNTLYLQMNSLRAEDTAVFYCARAPNYIGAFDVWGQGTMVTVSSGGGGSGGGGSGGGGSDIQMTQSPSSLSASVGDRVTITCRASQGISSWLAWYQQKPEKAPKSLIYAASSLQSGVPSRFSGSGSGTDFTLTISSLQPEDFATYYCQQYNSYPPTFGQGTKVEIK

SEQ ID NO: 79 - protein, 246 aa, synthetic construct
  source 1..246: note = CD80 extracellular domain
MGHTRRQGTSPSKCPYLNFFQLLVLAGLSHFCSGVIHVTKEVKEVATLSCGHNVSVEELAQTRIYWQKEKKMVLTMMSGDMNIWPEYKNRTIFDITNNLSIVILALRPSDEGTYECVVLKYEKDAFKREHLAEVTLSVKADFPTPSISDFEIPTSNIRRIICSTSGGFPEPHLSWLENGEELNAINTTVSQDPETELYAVSSKLDFNMTTNHSFMCLIKYGHLRVNQTFNWNTTKQEHFPDNLLPS

SEQ ID NO: 80 - protein, 232 aa, synthetic construct
  source 1..232: note = CD86 extracellular domain
FVMAFLLSGAAPLKIQAYFNETADLPCQFANSQNQSLSELVVFWQDQENLVLNEVYLGKEKFDSVHSKYMGRTSFDSDSWTLRLHNLQIKDKGLYQCIIHHKKPTGMIRIHQMNSELSVLANFSQPEIVPISNITENVYINLTCSSIHGYPEPKKMSVLLRTKNSTIEYDGVMQKSQDNVTELYDVSISLSVSFPDVTSNMTIFCILETDKTRLLSSPFSIELEDPQPPPDH

SEQ ID NO: 81 - protein, 22 aa, synthetic construct
  source 1..22: note = CD80 transmembrane domain
WAITLISVNGIFVICCLTYCFA

SEQ ID NO: 82 - protein, 23 aa, synthetic construct
  source 1..23: note = CD86 transmembrane domain
IPWITAVLPTVIICVMVFCLILW